European Patent Specification EP 3 682 000 B1, published April 5, 2023. Title: A gRNA TARGETING HPK1 AND A METHOD FOR EDITING HPK1 GENE. Applicant: Tsinghua University. The sequence listing filed with the application follows.

SEQUENCE LISTING (19 sequences)

SEQ ID NO: 1 - DNA, 19 bp, Artificial Sequence
gacctggtggcactgaaga

SEQ ID NO: 2 - DNA, 20 bp, Artificial Sequence
ggccaggatggttcttaggt

SEQ ID NO: 3 - DNA, 23 bp, Artificial Sequence
tagggacctggtggcactgaaga

SEQ ID NO: 4 - DNA, 23 bp, Artificial Sequence
aaactcttcagtgccaccaggtc

SEQ ID NO: 5 - DNA, 24 bp, Artificial Sequence
taggggccaggatggttcttaggt

SEQ ID NO: 6 - DNA, 24 bp, Artificial Sequence
aaacacctaagaaccatcctggcc

SEQ ID NO: 7 - DNA, 19 bp, Artificial Sequence
agcgagagtgaggaggggg

SEQ ID NO: 8 - DNA, 22 bp, Artificial Sequence
ttcatcaccagagataactccc

SEQ ID NO: 9 - DNA, 39 bp, Artificial Sequence
ccaccctctccccagtcctaccccctcctcacccctcct

SEQ ID NO: 10 - DNA, 39 bp, Artificial Sequence
ggtccctccagacccctcgctccgggacccctgggctgc

SEQ ID NO: 11 - DNA, 19 bp, Artificial Sequence
gctcgagacaaggtgtcag

SEQ ID NO: 12 - DNA, 19 bp, Artificial Sequence
aaggtgtcaggggacctgg

SEQ ID NO: 13 - DNA, 20 bp, Artificial Sequence
accactatgacctgctacag

SEQ ID NO: 14 - DNA, 20 bp, Artificial Sequence
gacctgctacagcggctggg

SEQ ID NO: 15 - DNA, 20 bp, Artificial Sequence
gctgggtggcggcacgtatg

SEQ ID NO: 16 - DNA, 2819 bp, human
agcgagagtgaggaggggggaggccacagcccgcggaggcaaggcgggtgcagggcttctggggacggagggaggtgccagaagttgagccctgaggccctgctggcccctgggcgcaggcccagctcaggcccccagggatggacgtcgtggaccctgacattttcaatagagacccccgggaccactatgacctgctacagcggctgggtggcggcacgtatggggaagtctttaaggctcgagacaaggtgtcaggggacctggtggcactgaagatggtgaagatggagcctgatgatgatgtctccacccttcagaaggaaatcctcatattgaaaacttgccggcacgccaacatcgtggcctaccatgggagttatctctggttgcagaaactctggatctgcatggaattctgtggggctggttctctccaggacatctaccaagtgacaggctccctgtcagagctccagattagctatgtctgccgggaagtgctccagggactggcctatttgcactcacagaagaagatacacagggacatcaagggagctaacatcctcatcaatgatgctggggaggtcagattggctgactttggcatctcggcccagattggggctacactggccagacgcctctctttcattgggacaccctactggatggctccggaagtggcagctgtggccctgaagggaggatacaatgagctgtgtgacatctggtccctgggcatcacggccatcgaactggccgagctacagccaccgctctttgatgtgcaccctctcagagttctcttcctcatgaccaagagtggctaccagcctccccgactgaaggaaaaaggcaaatggtcggctgccttccacaacttcatcaaagtcactctgactaagagtcccaagaaacgacccagcgccaccaagatgctcagtcatcaactggtatcccagcctgggctgaatcgaggcctgatcctggatcttcttgacaaactgaagaatcccgggaaaggaccctccattggggacattgaggatgaggagcccgagctaccccctgctatccctcggcggatcagatccacccaccgctccagctctctggggatcccagatgcagactgctgtcggcggcacatggagttcaggaagctccgaggaatggagaccagacccccagccaacaccgctcgcctacagcctcctcgagacctcaggagcagcagccccaggaagcaactgtcagagtcgtctgacgatgactatgacgacgtggacatccccacccctgcagaggacacacctcctccacttccccccaagcccaagttccgttctccatcagacgagggtcctgggagcatgggggatgatgggcagctgagcccgggggtgctggtccggtgtgccagtgggcccccaccaaacagcccccgtcctgggcctcccccatccaccagcagcccccacctcaccgcccattcagaaccctcactctggaacccaccctcccgggagcttgacaagcccccacttctgccccccaagaaggaaaagatgaagagaaagggatgtgcccttctcgtaaagttgttcaatggctgccccctccggatccacagcacggccgcctggacacatccctccaccaaggaccagcacctgctcctgggggcagaggaaggcatcttcatcctgaaccggaatgaccaggaggccacgctggaaatgctctttcctagccggactacgtgggtgtactccatcaacaacgttctcatgtctctctcaggaaagaccccccacctgtattctcatagcatccttggcctgctggaacggaaagagaccagagcaggaaaccccatcgctcacattagcccccaccgcctactggcaaggaagaacatggtttccaccaagatccaggacaccaaaggctgccgggcgtgctgtgtggcggagggtgcgagctctgggggcccgttcctgtgcggtgcattggagacgtccgttgtcctgcttcagtggtaccagcccatgaacaaattcctgcttgtccggcaggtgctgttcccactgccgacgcctctgtccgtgttcgcgctgctgaccgggccaggctctgagctgcccgctgtgtgcatcggcgtgagccccgggcggccggggaagtcggtgctcttccacacggtgcgctttggcgcgctctcttgctggctgggcgagatgagcaccgagcacaggggacccgtgcaggtgacccaggtagaggaagatatggtgatggtgttgatggatggctctgtgaagctggtgaccccggaggggtccccagtccggggacttcgcacacctgagatccccatgaccgaagcggtggaggccgtggctatggttggaggtcagcttcaggccttctggaagcatggagtgcaggtgtgggctctaggctcggatcagctgctacaggagctgagagaccctaccctcactttccgtctgcttggctcccccaggctggagtgcagtggcacgatctcgcctcactgcaacctcctcctcccaggttcaagcaattctcctgcctcagcctcccgagtagctgggattacaggcctgtagtggtggagacacgcccagtggatgatcctactgctcccagcaacctctacatccaggaatgagtccctaggggggtgtcaggaactagtccttgcaccccctcccccatagacacactagtggtcatggcatgtcctcatctcccaataaacatgactttagcctctgctaaaaaaa

SEQ ID NO: 17 - DNA, 2721 bp, human
agcgagagtgaggaggggggaggccacagcccgcggaggcaaggcgggtgcagggcttctggggacggagggaggtgccagaagttgagccctgaggccctgctggcccctgggcgcaggcccagctcaggcccccagggatggacgtcgtggaccctgacattttcaatagagacccccgggaccactatgacctgctacagcggctgggtggcggcacgtatggggaagtctttaaggctcgagacaaggtgtcaggggacctggtggcactgaagatggtgaagatggagcctgatgatgatgtctccacccttcagaaggaaatcctcatattgaaaacttgccggcacgccaacatcgtggcctaccatgggagttatctctggttgcagaaactctggatctgcatggaattctgtggggctggttctctccaggacatctaccaagtgacaggctccctgtcagagctccagattagctatgtctgccgggaagtgctccagggactggcctatttgcactcacagaagaagatacacagggacatcaagggagctaacatcctcatcaatgatgctggggaggtcagattggctgactttggcatctcggcccagattggggctacactggccagacgcctctctttcattgggacaccctactggatggctccggaagtggcagctgtggccctgaagggaggatacaatgagctgtgtgacatctggtccctgggcatcacggccatcgaactggccgagctacagccaccgctctttgatgtgcaccctctcagagttctcttcctcatgaccaagagtggctaccagcctccccgactgaaggaaaaaggcaaatggtcggctgccttccacaacttcatcaaagtcactctgactaagagtcccaagaaacgacccagcgccaccaagatgctcagtcatcaactggtatcccagcctgggctgaatcgaggcctgatcctggatcttcttgacaaactgaagaatcccgggaaaggaccctccattggggacattgaggatgaggagcccgagctaccccctgctatccctcggcggatcagatccacccaccgctccagctctctggggatcccagatgcagactgctgtcggcggcacatggagttcaggaagctccgaggaatggagaccagacccccagccaacaccgctcgcctacagcctcctcgagacctcaggagcagcagccccaggaagcaactgtcagagtcgtctgacgatgactatgacgacgtggacatccccacccctgcagaggacacacctcctccacttccccccaagcccaagttccgttctccatcagacgagggtcctgggagcatgggggatgatgggcagctgagcccgggggtgctggtccggtgtgccagtgggcccccaccaaacagcccccgtcctgggcctcccccatccaccagcagcccccacctcaccgcccattcagaaccctcactctggaacccaccctcccgggagcttgacaagcccccacttctgccccccaagaaggaaaagatgaagagaaagggatgtgcccttctcgtaaagttgttcaatggctgccccctccggatccacagcacggccgcctggacacatccctccaccaaggaccagcacctgctcctgggggcagaggaaggcatcttcatcctgaaccggaatgaccaggaggccacgctggaaatgctctttcctagccggactacgtgggtgtactccatcaacaacgttctcatgtctctctcaggaaagaccccccacctgtattctcatagcatccttggcctgctggaacggaaagagaccagagcaggaaaccccatcgctcacattagcccccaccgcctactggcaaggaagaacatggtttccaccaagatccaggacaccaaaggctgccgggcgtgctgtgtggcggagggtgcgagctctgggggcccgttcctgtgcggtgcattggagacgtccgttgtcctgcttcagtggtaccagcccatgaacaaattcctgcttgtccggcaggtgctgttcccactgccgacgcctctgtccgtgttcgcgctgctgaccgggccaggctctgagctgcccgctgtgtgcatcggcgtgagccccgggcggccggggaagtcggtgctcttccacacggtgcgctttggcgcgctctcttgctggctgggcgagatgagcaccgagcacaggggacccgtgcaggtgacccaggtagaggaagatatggtgatggtgttgatggatggctctgtgaagctggtgaccccggaggggtccccagtccggggacttcgcacacctgagatccccatgaccgaagcggtggaggccgtggctatggttggaggtcagcttcaggccttctggaagcatggagtgcaggtgtgggctctaggctcggatcagctgctacaggagctgagagaccctaccctcactttccgtctgcttggctcccccaggcctgtagtggtggagacacgcccagtggatgatcctactgctcccagcaacctctacatccaggaatgagtccctaggggggtgtcaggaactagtccttgcaccccctcccccatagacacactagtggtcatggcatgtcctcatctcccaataaacatgactttagcctctgctaaaaaaa

SEQ ID NO: 18 - DNA, 4206 bp, Artificial Sequence
atggccccaaagaagaagcggaaggtcggtatccacggtgtcccagcagccatggacaagaagtactccattgggctcgatatcggcacaaacagcgtcggctgggccgtcattacggacgagtacaaggtgccgagcaaaaaattcaaagttctgggcaataccgatcgccacagcataaagaagaacctcattggcgccctcctgttcgactccggggagacggccgaagccacgcggctcaaaagaacagcacggcgcagatatacccgcagaaagaatcggatctgctacctgcaggagatctttagtaatgagatggctaaggtggatgactctttcttccataggctggaggagtcctttttggtggaggaggataaaaagcacgagcgccacccaatctttggcaatatcgtggacgaggtggcgtaccatgaaaagtacccaaccatatatcatctgaggaagaagcttgtagacagtactgataaggctgacttgcggttgatctatctcgcgctggcgcatatgatcaaatttcggggacacttcctcatcgagggggacctgaacccagacaacagcgatgtcgacaaactctttatccaactggttcagacttacaatcagcttttcgaagagaacccgatcaacgcatccggagttgacgccaaagcaatcctgagcgctaggctgtccaaatcccggcggctcgaaaacctcatcgcacagctccctggggagaagaagaacggcctgtttggtaatcttatcgccctgtcactcgggctgacccccaactttaaatctaacttcgacctggccgaagatgccaagcttcaactgagcaaagacacctacgatgatgatctcgacaatctgctggcccagatcggcgaccagtacgcagacctttttttggcggcaaagaacctgtcagacgccattctgctgagtgatattctgcgagtgaacacggagatcaccaaagctccgctgagcgctagtatgatcaagcgctatgatgagcaccaccaagacttgactttgctgaaggcccttgtcagacagcaactgcctgagaagtacaaggaaattttcttcgatcagtctaaaaatggctacgccggatacattgacggcggagcaagccaggaggaattttacaaatttattaagcccatcttggaaaaaatggacggcaccgaggagctgctggtaaagcttaacagagaagatctgttgcgcaaacagcgcactttcgacaatggaagcatcccccaccagattcacctgggcgaactgcacgctatactcaggcggcaagaggatttctacccctttttgaaagataacagggaaaagattgagaaaatcctcacatttcggataccctactatgtaggccccctcgcccggggaaattccagattcgcgtggatgactcgcaaatcagaagagaccatcactccctggaacttcgaggaagtcgtggataagggggcctctgcccagtccttcatcgaaaggatgactaactttgataaaaatctgcctaacgaaaaggtgcttcctaaacactctctgctgtacgagtacttcacagtttataacgagctcaccaaggtcaaatacgtcacagaagggatgagaaagccagcattcctgtctggagagcagaagaaagctatcgtggacctcctcttcaagacgaaccggaaagttaccgtgaaacagctcaaagaagactatttcaaaaagattgaatgtttcgactctgttgaaatcagcggagtggaggatcgcttcaacgcatccctgggaacgtatcacgatctcctgaaaatcattaaagacaaggacttcctggacaatgaggagaacgaggacattcttgaggacattgtcctcacccttacgttgtttgaagatagggagatgattgaagaacgcttgaaaacttacgctcatctcttcgacgacaaagtcatgaaacagctcaagaggcgccgatatacaggatgggggcggctgtcaagaaaactgatcaatgggatccgagacaagcagagtggaaagacaatcctggattttcttaagtccgatggatttgccaaccggaacttcatgcagttgatccatgatgactctctcacctttaaggaggacatccagaaagcacaagtttctggccagggggacagtcttcacgagcacatcgctaatcttgcaggtagcccagctatcaaaaagggaatactgcagaccgttaaggtcgtggatgaactcgtcaaagtaatgggaaggcataagcccgagaatatcgttatcgagatggcccgagagaaccaaactacccagaagggacagaagaacagtagggaaaggatgaagaggattgaagagggtataaaagaactggggtcccaaatccttaaggaacacccagttgaaaacacccagcttcagaatgagaagctctacctgtactacctgcagaacggcagggacatgtacgtggatcaggaactggacatcaatcggctctccgactacgacgtggatcatatcgtgccccagtcttttctcaaagatgattctattgataataaagtgttgacaagatccgataaaaatagagggaagagtgataacgtcccctcagaagaagttgtcaagaaaatgaaaaattattggcggcagctgctgaacgccaaactgatcacacaacggaagttcgataatctgactaaggctgaacgaggtggcctgtctgagttggataaagcaggcttcatcaaaaggcagcttgttgagacacgccagatcaccaagcacgtggcccaaattctcgattcacgcatgaacaccaagtacgatgaaaatgacaaactgattcgagaggtgaaagttattactctgaagtctaagctggtctcagatttcagaaaggactttcagttttataaggtgagagagatcaacaattaccaccatgcgcatgatgcctacctgaatgcagtggtaggcactgcacttatcaaaaaatatcccaagcttgaatctgaatttgtttacggagactataaagtgtacgatgttaggaaaatgatcgcaaagtctgagcaggaaataggcaaggccaccgctaagtacttcttttacagcaatattatgaattttttcaagaccgagattacactggccaatggagagattcggaagcgaccacttatcgaaacaaacggagaaacaggagaaatcgtgtgggacaagggtagggatttcgcgacagtccggaaggtcctgtccatgccgcaggtgaacatcgttaaaaagaccgaagtacagaccggaggcttctccaaggaaagtatcctcccgaaaaggaacagcgacaagctgatcgcacgcaaaaaagattgggaccccaagaaatacggcggattcgattctcctacagtcgcttacagtgtactggttgtggccaaagtggagaaagggaagtctaaaaaactcaaaagcgtcaaggaactgctgggcatcacaatcatggagcgatcaagcttcgaaaaaaaccccatcgactttctcgaggcgaaaggatataaagaggtcaaaaaagacctcatcattaagcttcccaagtactctctctttgagcttgaaaacggccggaaacgaatgctcgctagtgcgggcgagctgcagaaaggtaacgagctggcactgccctctaaatacgttaatttcttgtatctggccagccactatgaaaagctcaaagggtctcccgaagataatgagcagaagcagctgttcgtggaacaacacaaacactaccttgatgagatcatcgagcaaataagcgaattctccaaaagagtgatcctcgccgacgctaacctcgataaggtgctttctgcttacaataagcacagggataagcccatcagggagcaggcagaaaacattatccacttgtttactctgaccaacttgggcgcgcctgcagccttcaagtacttcgacaccaccatagacagaaagcggtacacctctacaaaggaggtcctggacgccacactgattcatcagtcaattacggggctctatgaaacaagaatcgacctctctcagctcggtggagacaagcgtcctgctgctactaagaaagctggtcaagctaagaaaaagaaataa

SEQ ID NO: 19 - protein, 1401 aa, Artificial Sequence [sequence omitted]